European Patent Application EP 4 725 962 A1, published April 15, 2026. Title: Process and device for cultivation of iPSC. Applicant: Gottfried Wilhelm Leibniz Universität Hannover. The sequence listing filed with the application follows.

SEQUENCE LISTING (38 sequences)

SEQ ID NO: 1 - protein, 15 aa, synthetic construct
WLSERPKLAPDAEDS

SEQ ID NO: 2 - protein, 15 aa, synthetic construct
HTQSTSVDTNNPIYV

SEQ ID NO: 3 - protein, 15 aa, synthetic construct
YMGSRQATGDYMGVS

SEQ ID NO: 4 - protein, 15 aa, synthetic construct
KASRRSRQPARHPAC

SEQ ID NO: 5 - protein, 15 aa, synthetic construct
RQHQGAEHPQPHTLF

SEQ ID NO: 6 - protein, 15 aa, synthetic construct
SKAIQVFLLGGSRKR

SEQ ID NO: 7 - protein, 12 aa, synthetic construct
ASKAIQVFLLGG

SEQ ID NO: 8 - protein, 15 aa, synthetic construct
ASIKVAVSADRDCIR

SEQ ID NO: 9 - protein, 15 aa, synthetic construct
SGSTRLEFPDFPIDD

SEQ ID NO: 10 - protein, 15 aa, synthetic construct
GGQIKKSPAVKVTHF

SEQ ID NO: 11 - protein, 15 aa, synthetic construct
ITLLTDRRYNNGTWY

SEQ ID NO: 12 - protein, 15 aa, synthetic construct
FATTNSSGIILAALG

SEQ ID NO: 13 - protein, 15 aa, synthetic construct
HSISLVRNRRIITVQ

SEQ ID NO: 14 - protein, 15 aa, synthetic construct
PVEMKLGTLVESRTI

SEQ ID NO: 15 - protein, 15 aa, synthetic construct
ESRTINVSNLYVGGI

SEQ ID NO: 16 - protein, 15 aa, synthetic construct
QYQARKIGNITHSIP

SEQ ID NO: 17 - protein, 15 aa, synthetic construct
VNITLEFRTSSQNGV

SEQ ID NO: 18 - protein, 15 aa, synthetic construct
GSGSGSGELIAQARG

SEQ ID NO: 19 - protein, 15 aa, synthetic construct
AQARGAASKVKVPMK

SEQ ID NO: 20 - protein, 15 aa, synthetic construct
GVQLRTPRDLADLAA

SEQ ID NO: 21 - protein, 15 aa, synthetic construct
GPAVLSIDEDIGEQF

SEQ ID NO: 22 - protein, 15 aa, synthetic construct
PPSLRRLFPTGGSVR

SEQ ID NO: 23 - protein, 15 aa, synthetic construct
TGNVYSGFGFHSAQD

SEQ ID NO: 24 - protein, 15 aa, synthetic construct
MKPHRGPPPELQPQP

SEQ ID NO: 25 - protein, 15 aa, synthetic construct
RHPACMLPPHLRTTR

SEQ ID NO: 26 - protein, 15 aa, synthetic construct
GGSLSSHLEFVGILA

SEQ ID NO: 27 - protein, 15 aa, synthetic construct
VGILARHRNWPSLSM

SEQ ID NO: 28 - protein, 15 aa, synthetic construct
SSRGLLLFTARLRPG

SEQ ID NO: 29 - protein, 15 aa, synthetic construct
QMEGLGTRLRAQSRQ

SEQ ID NO: 30 - protein, 15 aa, synthetic construct
TVGFSGCVKRLRLHG

SEQ ID NO: 31 - protein, 15 aa, synthetic construct
FPGSGGVITLDLPGA

SEQ ID NO: 32 - protein, 15 aa, synthetic construct
GLELEVRPLAVTGLI

SEQ ID NO: 33 - protein, 15 aa, synthetic construct
VTGLIFHLGQARTPP

SEQ ID NO: 34 - protein, 15 aa, synthetic construct
DDGAGEFSTSVTRPS

SEQ ID NO: 35 - protein, 15 aa, synthetic construct
QWHRLAVMKSGNVLR

SEQ ID NO: 36 - protein, 15 aa, synthetic construct
YLGGLPEPMAVQPWP

SEQ ID NO: 37 - protein, 15 aa, synthetic construct
LQPPPPLTSASKAIQ

SEQ ID NO: 38 - protein, 15 aa, synthetic construct
LLISQARKQAASIKV